European Patent Application EP 4 635 974 A1, published October 22, 2025. Title: 피부 개선용 화장료 조성물. Applicant: 주식회사 엘지생활건강. Application KR. The sequence listing filed with the application follows.

SEQUENCE LISTING (19 sequences)

SEQ ID NO: 1 - protein, 10 aa, synthetic construct
KGRSSCFVDC

SEQ ID NO: 2 - protein, 9 aa, synthetic construct
KGRSSCFVD

SEQ ID NO: 3 - protein, 7 aa, synthetic construct
KGRSSCF

SEQ ID NO: 4 - protein, 8 aa, synthetic construct
KGRSSCFV

SEQ ID NO: 5 - protein, 8 aa, synthetic construct
RSSCFVDC

SEQ ID NO: 6 - protein, 7 aa, synthetic construct
SSCFVDC

SEQ ID NO: 7 - protein, 8 aa, synthetic construct
GRSSCFVD

SEQ ID NO: 8 - protein, 7 aa, synthetic construct
RSSCFVD

SEQ ID NO: 9 - protein, 6 aa, synthetic construct
SSCFVD

SEQ ID NO: 10 - protein, 9 aa, synthetic construct
KGSSCFVDC

SEQ ID NO: 11 - protein, 9 aa, synthetic construct
KGRSSCFDC

SEQ ID NO: 12 - protein, 9 aa, synthetic construct
KGRSSCFVC

SEQ ID NO: 13 - protein, 5 aa, synthetic construct
RSSCF

SEQ ID NO: 14 - protein, 10 aa, synthetic construct
CDVFCSSRGK

SEQ ID NO: 15 - protein, 9 aa, synthetic construct
DVFCSSRGK

SEQ ID NO: 16 - protein, 7 aa, synthetic construct
FCSSRGK

SEQ ID NO: 17 - DNA, 30 bp, synthetic construct
  source 1..30: mol_type = other DNA
aaaggccgcagcagctgctttgtggattgc

SEQ ID NO: 18 - DNA, 27 bp, synthetic construct
  source 1..27: mol_type = other DNA
aaaggccgcagcagctgctttgtggat

SEQ ID NO: 19 - DNA, 21 bp, synthetic construct
  source 1..21: mol_type = other DNA
aaaggccgcagcagctgcttt